European Patent Application EP 4 640 237 A2, published October 29, 2025. Title: Macrophage-based Therapy. Applicant: The University Court of the University of Edinburgh. The sequence listing filed with the application follows.

SEQUENCE LISTING (24 sequences)

SEQ ID NO: 1 - DNA, 19 bp, synthetic construct
  misc_feature 1..19: note = iNOS forward primer
  source 1..19: mol_type = other DNA
aacacccgggacatgagac

SEQ ID NO: 2 - DNA, 20 bp, synthetic construct
  misc_feature 1..20: note = iNOS reverse primer
  source 1..20: mol_type = other DNA
cctgggaggatcaggaagtc

SEQ ID NO: 3 - DNA, 19 bp, synthetic construct
  misc_feature 1..19: note = CD86 forward primer
  source 1..19: mol_type = other DNA
gaagccgaatcagcctagc

SEQ ID NO: 4 - DNA, 20 bp, synthetic construct
  misc_feature 1..20: note = CD86 reverse primer
  source 1..20: mol_type = other DNA
cagcgttactatcccgctct

SEQ ID NO: 5 - DNA, 18 bp, synthetic construct
  misc_feature 1..18: note = ARG1 forward primer
  source 1..18: mol_type = other DNA
gaatctgcatgggcaacc

SEQ ID NO: 6 - DNA, 22 bp, synthetic construct
  misc_feature 1..22: note = ARG1 reverse primer
  source 1..22: mol_type = other DNA
gaatcctggtacatctgggaac

SEQ ID NO: 7 - DNA, 20 bp, synthetic construct
  misc_feature 1..20: note = FIZZ1 forward primer
  source 1..20: mol_type = other DNA
tatgaacagatgggcctcct

SEQ ID NO: 8 - DNA, 21 bp, synthetic construct
  misc_feature 1..21: note = FIZZ1 reverse primer
  source 1..21: mol_type = other DNA
aggcagttgcaagtatctcca

SEQ ID NO: 9 - DNA, 19 bp, synthetic construct
  misc_feature 1..19: note = TWEAK forward primer
  source 1..19: mol_type = other DNA
caggatggagcacaagcag

SEQ ID NO: 10 - DNA, 20 bp, synthetic construct
  misc_feature 1..20: note = TWEAK reverse primer
  source 1..20: mol_type = other DNA
ggctggagctgttgattttg

SEQ ID NO: 11 - DNA, 19 bp, synthetic construct
  misc_feature 1..19: note = MMP9 forward primer
  source 1..19: mol_type = other DNA
acgacatagacggcatcca

SEQ ID NO: 12 - DNA, 20 bp, synthetic construct
  misc_feature 1..20: note = MMP9 reverse primer
  source 1..20: mol_type = other DNA
gctgtggttcagttgtggtg

SEQ ID NO: 13 - DNA, 19 bp, synthetic construct
  misc_feature 1..19: note = MMP12 forward primer
  source 1..19: mol_type = other DNA
gctgctcccatgaatgaca

SEQ ID NO: 14 - DNA, 20 bp, synthetic construct
  misc_feature 1..20: note = MMP12 reverse primer
  source 1..20: mol_type = other DNA
aagcattgcacacggttgta

SEQ ID NO: 15 - DNA, 19 bp, synthetic construct
  misc_feature 1..19: note = MMP13 forward primer
  source 1..19: mol_type = other DNA
gccagaacttcccaaccat

SEQ ID NO: 16 - DNA, 21 bp, synthetic construct
  misc_feature 1..21: note = MMP13 reverse primer
  source 1..21: mol_type = other DNA
tcagagcccagaattttctcc

SEQ ID NO: 17 - DNA, 20 bp, synthetic construct
  misc_feature 1..20: note = CD40 forward primer
  source 1..20: mol_type = other DNA
gccaagaagccaaccaataa

SEQ ID NO: 18 - DNA, 21 bp, synthetic construct
  misc_feature 1..21: note = CD40 reverse primer
  source 1..21: mol_type = other DNA
tggcatccatgtaaagtctcc

SEQ ID NO: 19 - DNA, 20 bp, synthetic construct
  misc_feature 1..20: note = CD80 forward primer
  source 1..20: mol_type = other DNA
aagcaaggggctgaaaagat

SEQ ID NO: 20 - DNA, 19 bp, synthetic construct
  misc_feature 1..19: note = CD80 reverse primer
  source 1..19: mol_type = other DNA
aagggcaaggtggggtaat

SEQ ID NO: 21 - DNA, 20 bp, synthetic construct
  misc_feature 1..20: note = TGM2 forward primer
  source 1..20: mol_type = other DNA
tcaccttcagtgtcgtgacc

SEQ ID NO: 22 - DNA, 22 bp, synthetic construct
  misc_feature 1..22: note = TGM2 reverse primer
  source 1..22: mol_type = other DNA
cagcatctcttagtggaaaacg

SEQ ID NO: 23 - DNA, 20 bp, synthetic construct
  misc_feature 1..20: note = MRC1 forward primer
  source 1..20: mol_type = other DNA
tgttttggttgggattgaca

SEQ ID NO: 24 - DNA, 21 bp, synthetic construct
  misc_feature 1..21: note = MRC1 reverse primer
  source 1..21: mol_type = other DNA
tctccataagcccagttttca